European Patent Application EP 4 494 658 A1, published January 22, 2025. Title: 抗体药物偶联物及其应用. Applicant: 上海华奥泰生物药业股份有限公司. The sequence listing filed with the application follows.

SEQUENCE LISTING (54 sequences)

SEQ ID NO: 1 - protein, 8 aa, synthetic construct
  REGION 1..8: note = 900581, 900694, 900695, 900696, 900697, 900698 (HCDR1)
GFTFSKYA

SEQ ID NO: 2 - protein, 8 aa, synthetic construct
  REGION 1..8: note = 900581, 900694, 900695, 900696, 900697, 900698 (HCDR2)
ISSGGGYI

SEQ ID NO: 3 - protein, 18 aa, synthetic construct
  REGION 1..18: note = 900581, 900694, 900695, 900696, 900697, 900698 (HCDR3)
ARAIYYYGSSYNYYAMDY

SEQ ID NO: 4 - protein, 6 aa, synthetic construct
  REGION 1..6: note = 900581, 900694, 900695, 900696, 900697, 900698 (LCDR1)
QDVGTA

SEQ ID NO: 5 - skipped

SEQ ID NO: 6 - protein, 9 aa, synthetic construct
  REGION 1..9: note = 900581, 900694, 900695, 900696, 900697, 900698 (LCDR3)
QQYSSYPLT

SEQ ID NO: 7 - protein, 25 aa, synthetic construct
  REGION 1..25: note = 900581 (H-FR1)
EVQLVESGGGLVKPGGSLKLSCAAS

SEQ ID NO: 8 - protein, 17 aa, synthetic construct
  REGION 1..17: note = 900581 (H-FR2)
MSWVRQSPEKRLEWVAE

SEQ ID NO: 9 - protein, 38 aa, synthetic construct
  REGION 1..38: note = 900581 (H-FR3)
NYPDTVTGRFTISRDNAKNTLYLEMSSLRSGDTAMYYC

SEQ ID NO: 10 - protein, 11 aa, synthetic construct
  REGION 1..11: note = 900581 (H-FR4)
WGQGTSVTVSS

SEQ ID NO: 11 - protein, 26 aa, synthetic construct
  REGION 1..26: note = 900581 (L-FR1)
DIVMTQSHKFMSTSVGDRVSITCKAS

SEQ ID NO: 12 - protein, 17 aa, synthetic construct
  REGION 1..17: note = 900581 (L-FR2)
EAWYQQKPGQSPKLLIY

SEQ ID NO: 13 - protein, 36 aa, synthetic construct
  REGION 1..36: note = 900581 (L-FR3)
TRHTGVPDRFTGSGSGTDFTLTIGNVQSEDLADYFC

SEQ ID NO: 14 - protein, 10 aa, synthetic construct
  REGION 1..10: note = 900581 (L-FR4)
FGGGTKLEIK

SEQ ID NO: 15 - protein, 25 aa, synthetic construct
  REGION 1..25: note = 900694 (H-FR1)
EVQLVESGGGLVKPGGSLRLSCAAS

SEQ ID NO: 16 - protein, 17 aa, synthetic construct
  REGION 1..17: note = 900694, 900695, 900697 (H-FR2)
MSWVRQAPGKGLEWVAE

SEQ ID NO: 17 - protein, 38 aa, synthetic construct
  REGION 1..38: note = 900694 (H-FR3)
NYPDTVTGRFTISRDNAKNSLYLQMNSLRAEDTAVYYC

SEQ ID NO: 18 - protein, 11 aa, synthetic construct
  REGION 1..11: note = 900694, 900695, 900696, 900697, 900698 (H-FR4)
WGQGTTVTVSS

SEQ ID NO: 19 - protein, 25 aa, synthetic construct
  REGION 1..25: note = 900695, 900697, 900696, 900698 (H-FR1)
QVQLVESGGGLVKPGGSLRLSCAAS

SEQ ID NO: 20 - protein, 38 aa, synthetic construct
  REGION 1..38: note = 900695, 900697(H-FR3)
NYADSVTGRFTISRDNAKNSLYLQMNSLRAEDTAVYYC

SEQ ID NO: 21 - protein, 17 aa, synthetic construct
  REGION 1..17: note = 900696, 900698(H-FR2)
MSWIRQAPGKGLEWVAE

SEQ ID NO: 22 - protein, 38 aa, synthetic construct
  REGION 1..38: note = 900696, 900698(H-FR3)
NYADSVKGRFTISRDNAKNSLYLQMNSLRAEDTAVYYC

SEQ ID NO: 23 - protein, 26 aa, synthetic construct [sequence omitted]

SEQ ID NO: 24 - protein, 17 aa, synthetic construct
  REGION 1..17: note = 900694, 900695, 900696, 900697, 900698 (L-FR2)
EAWYQQKPGKAPKLLIY

SEQ ID NO: 25 - protein, 36 aa, synthetic construct
  REGION 1..36: note = 900694 (L-FR3)
TRHTGVPDRFSGSGSGTDFTLTISSLQPEDFATYYC

SEQ ID NO: 26 - protein, 10 aa, synthetic construct
  REGION 1..10: note = 900694, 900695, 900696, 900697, 900698 (L-FR4)
FGQGTKLEIK

SEQ ID NO: 27 - protein, 36 aa, synthetic construct
  REGION 1..36: note = 900695, 900698 (L-FR3)
TRHTGVPSRFSGSGSGTDFTLTISSLQPEDFATYYC

SEQ ID NO: 28 - protein, 36 aa, synthetic construct
  REGION 1..36: note = 900696, 900697 (L-FR3)
TLQSGVPSRFSGSGSGTDFTLTISSLQPEDFATYYC

SEQ ID NO: 29 - protein, 125 aa, synthetic construct
  REGION 1..125: note = 900581 (VH)
EVQLVESGGGLVKPGGSLKLSCAASGFTFSKYAMSWVRQSPEKRLEWVAEISSGGGYINYPDTVTGRFTISRDNAKNTLYLEMSSLRSGDTAMYYCARAIYYYGSSYNYYAMDYWGQGTSVTVSS

SEQ ID NO: 30 - protein, 107 aa, synthetic construct
  REGION 1..107: note = 900581 (VL)
DIVMTQSHKFMSTSVGDRVSITCKASQDVGTAEAWYQQKPGQSPKLLIYWASTRHTGVPDRFTGSGSGTDFTLTIGNVQSEDLADYFCQQYSSYPLTFGGGTKLEIK

SEQ ID NO: 31 - protein, 125 aa, synthetic construct
  REGION 1..125: note = 900694 (VH)
EVQLVESGGGLVKPGGSLRLSCAASGFTFSKYAMSWVRQAPGKGLEWVAEISSGGGYINYPDTVTGRFTISRDNAKNSLYLQMNSLRAEDTAVYYCARAIYYYGSSYNYYAMDYWGQGTTVTVSS

SEQ ID NO: 32 - protein, 107 aa, synthetic construct
  REGION 1..107: note = 900694 (VL)
DIQMTQSPSSLSASVGDRVTITCRASQDVGTAEAWYQQKPGKAPKLLIYWASTRHTGVPDRFSGSGSGTDFTLTISSLQPEDFATYYCQQYSSYPLTFGQGTKLEIK

SEQ ID NO: 33 - protein, 125 aa, synthetic construct
  REGION 1..125: note = 900695, 900697 (VH)
QVQLVESGGGLVKPGGSLRLSCAASGFTFSKYAMSWVRQAPGKGLEWVAEISSGGGYINYADSVTGRFTISRDNAKNSLYLQMNSLRAEDTAVYYCARAIYYYGSSYNYYAMDYWGQGTTVTVSS

SEQ ID NO: 34 - protein, 107 aa, synthetic construct
  REGION 1..107: note = 900695, 900698 (VL)
DIQMTQSPSSLSASVGDRVTITCRASQDVGTAEAWYQQKPGKAPKLLIYWASTRHTGVPSRFSGSGSGTDFTLTISSLQPEDFATYYCQQYSSYPLTFGQGTKLEIK

SEQ ID NO: 35 - protein, 125 aa, synthetic construct
  REGION 1..125: note = 900696, 900698 (VH)
QVQLVESGGGLVKPGGSLRLSCAASGFTFSKYAMSWIRQAPGKGLEWVAEISSGGGYINYADSVKGRFTISRDNAKNSLYLQMNSLRAEDTAVYYCARAIYYYGSSYNYYAMDYWGQGTTVTVSS

SEQ ID NO: 36 - protein, 107 aa, synthetic construct
  REGION 1..107: note = 900696, 900697 (VL)
DIQMTQSPSSLSASVGDRVTITCRASQDVGTAEAWYQQKPGKAPKLLIYWASTLQSGVPSRFSGSGSGTDFTLTISSLQPEDFATYYCQQYSSYPLTFGQGTKLEIK

SEQ ID NO: 37 - protein, 15 aa, synthetic construct
  REGION 1..15: note = CD73 (amino acid residues at position 143-157)
NIKAKGPLASQISGL

SEQ ID NO: 38 - protein, 14 aa, synthetic construct
  REGION 1..14: note = CD73 (amino acid residues at position178-191)
SKETPFLSNPGTNL

SEQ ID NO: 39 - protein, 6 aa, synthetic construct
  REGION 1..6: note = CD73 (amino acid residues at position 381-386)
WNHVSM

SEQ ID NO: 40 - protein, 574 aa, synthetic construct
  REGION 1..574: note = CD73 full-length sequence
MCPRAARAPATLLLALGAVLWPAAGAWELTILHTNDVHSRLEQTSEDSSKCVNASRCMGGVARLFTKVQQIRRAEPNVLLLDAGDQYQGTIWFTVYKGAEVAHFMNALRYDAMALGNHEFDNGVEGLIEPLLKEAKFPILSANIKAKGPLASQISGLYLPYKVLPVGDEVVGIVGYTSKETPFLSNPGTNLVFEDEITALQPEVDKLKTLNVNKIIALGHSGFEMDKLIAQKVRGVDVVVGGHSNTFLYTGNPPSKEVPAGKYPFIVTSDDGRKVPVVQAYAFGKYLGYLKIEFDERGNVISSHGNPILLNSSIPEDPSIKADINKWRIKLDNYSTQELGKTIVYLDGSSQSCRFRECNMGNLICDAMINNNLRHTDEMFWNHVSMCILNGGGIRSPIDERNNGTITWENLAAVLPFGGTFDLVQLKGSTLKKAFEHSVHRYGQSTGEFLQVGGIHVVYDLSRKPGDRVVKLDVLCTKCRVPSYDPLKMDEVYKVILPNFLANGGDGFQMIKDELLRHDSGDQDINVVSTYISKMKVIYPAVEGRIKFSTGSHCHGSFSLIFLSLWAVIFVLYQ

SEQ ID NO: 41 - protein, 122 aa, synthetic construct
  REGION 1..122: note = 900565 (VH)
QAYLQQSGAELVRPGASVKMSCKASGYTFTSYNMHWVKQTPRQGLEWIGAIYPGNGDTSYNQKFKGKATLNVDKSSSTAYMQLSSLTSEDSAVYFCARWGYGSNYAWYFDIWGTGTTVTVSS

SEQ ID NO: 42 - protein, 107 aa, synthetic construct
  REGION 1..107: note = 900565 (VL)
DIQMTQSPASLSASVGETVTITCRTSGNIHNYLVWYQQKQGKSPQLLVFNAKTLADGVPSRFSGSGSGTQYSLKINSLQPEDFGSYYCQHFWSTPFTFGSGTKLEIK

SEQ ID NO: 43 - protein, 450 aa, synthetic construct
  REGION 1..450: note = 900201 (HC)
QIQLVQSGPELKKPGETVKISCKTSGYTFTNYGMNWVKQAPGKGLKWVGWINTYTGEPKYADDFKGRFAFSVETSASTAYLQINNLKNEDTATYFCARGIYDGYHWYFDVWGAGTTVTVSSASTKGPSVFPLAPSSKSTSGGTAALGCLVKDYFPEPVTVSWNSGALTSGVHTFPAVLQSSGLYSLSSVVTVPSSSLGTQTYICNVNHKPSNTKVDKRVEPKSCDKTHTCPPCPAPELLGGPSVFLFPPKPKDTLMISRTPEVTCVVVDVSHEDPEVKFNWYVDGVEVHNAKTKPREEQYNSTYRVVSVLTVLHQDWLNGKEYKCKVSNKALPAPIEKTISKAKGQPREPQVYTLPPSREEMTKNQVSLTCLVKGFYPSDIAVEWESNGQPENNYKTTPPVLDSDGSFFLYSKLTVDKSRWQQGNVFSCSVMHEALHNHYTQKSLSLSPG

SEQ ID NO: 44 - protein, 219 aa, synthetic construct
  REGION 1..219: note = 900201 (LC)
DVVMTQTPLSLPVSLGDQASISCRSSQSLVHSIGNTYLHWYLQKPGQSPKLLIYKVSNRFSGVPDRFSGSGSGTDFTLKITRVEAEDLGVYFCSQSTHVPFTFGSGTKLEIKRTVAAPSVFIFPPSDEQLKSGTASVVCLLNNFYPREAKVQWKVDNALQSGNSQESVTEQDSKDSTYSLSSTLTLSKADYEKHKVYACEVTHQGLSSPVTKSFNRGEC

SEQ ID NO: 45 - protein, 450 aa, synthetic construct
  REGION 1..450: note = 900543 heavy chain
QIQLVQSGPELKKPGETVKISCKTSGYTFTNYGMNWVKQAPGKGLKWVGWINTYTGEPKYADDFKGRFAFSVETSASTAYLQINNLKNEDTATYFCARGIYDGYHWYFDVWGAGTTVTVSSASTKGPSVFPLAPSSKSTSGGTAALGCLVKDYFPEPVTVSWNSGALTSGVHTFPAVLQSSGLYSLSSVVTVPSSSLGTQTYICNVNHKPSNTKVDKRVEPKSCDKTHTCPPCPAPEAAGGPSVFLFPPKPKDTLMISRTPEVTCVVVDVSHEDPEVKFNWYVDGVEVHNAKTKPREEQYNSTYRVVSVLTVLHQDWLNGKEYKCKVSNKALPAPIEKTISKAKGQPREPQVYTLPPSREEMTKNQVSLTCLVKGFYPSDIAVEWESNGQPENNYKTTPPVLDSDGSFFLYSKLTVDKSRWQQGNVFSCSVMHEALHNHYTQKSLSLSPG

SEQ ID NO: 46 - protein, 219 aa, synthetic construct; identical to SEQ ID NO: 44
  REGION 1..219: note = 900543 light chain

SEQ ID NO: 47 - protein, 447 aa, synthetic construct
  REGION 1..447: note = Oleclumab heavy chain
EVQLLESGGGLVQPGGSLRLSCAASGFTFSSYAYSWVRQAPGKGLEWVSAISGSGGRTYYADSVKGRFTISRDNSKNTLYLQMNSLRAEDTAVYYCARLGYGRVDEWGRGTLVTVSSASTKGPSVFPLAPSSKSTSGGTAALGCLVKDYFPEPVTVSWNSGALTSGVHTFPAVLQSSGLYSLSSVVTVPSSSLGTQTYICNVNHKPSNTKVDKRVEPKSCDKTHTCPPCPAPEFEGGPSVFLFPPKPKDTLMISRTPEVTCVVVDVSHEDPEVKFNWYVDGVEVHNAKTKPREEQYNSTYRVVSVLTVLHQDWLNGKEYKCKVSNKALPASIEKTISKAKGQPREPQVYTLPPSREEMTKNQVSLTCLVKGFYPSDIAVEWESNGQPENNYKTTPPVLDSDGSFFLYSKLTVDKSRWQQGNVFSCSVMHEALHNHYTQKSLSLSPGK

SEQ ID NO: 48 - protein, 216 aa, synthetic construct
  REGION 1..216: note = Oleclumab light chain
QSVLTQPPSASGTPGQRVTISCSGSLSNIGRNPVNWYQQLPGTAPKLLIYLDNLRLSGVPDRFSGSKSGTSASLAISGLQSEDEADYYCATWDDSHPGWTFGGGTKLTVLGQPKAAPSVTLFPPSSEELQANKATLVCLISDFYPGAVTVAWKADSSPVKAGVETTTPSKQSNNKYAASSYLSLTPEQWKSHRSYSCQVTHEGSTVEKTVAPTECS

SEQ ID NO: 49 - protein, 449 aa, synthetic construct
  REGION 1..449: note = Uliledlimab heavy chain
EVQLQESGPGLVKPSETLSLTCAVSGYSITSGYYWNWIRQPPGKKLEWMGYINYGGSNGYNPSLKSRITISRDTSKNQFSLKLSSVTAADTAVYYCARDYDAYYEALDDWGQGTTVTVSSASTKGPSVFPLAPSSKSTSGGTAALGCLVKDYFPEPVTVSWNSGALTSGVHTFPAVLQSSGLYSLSSVVTVPSSSLGTQTYICNVNHKPSNTKVDKRVEPKSCDKTHTCPPCPAPELLGGPSVFLFPPKPKDTLMISRTPEVTCVVVDVSHEDPEVKFNWYVDGVEVHNAKTKPREEQYNSTYRVVSVLTVLHQDWLNGKEYKCKVSNKALPAPIEKTISKAKGQPREPQVYTLPPSREEMTKNQVSLTCLVKGFYPSDIAVEWESNGQPENNYKTTPPVLDSDGSFFLYSKLTVDKSRWQQGNVFSCSVMHEALHNHYTQKSLSLSPG

SEQ ID NO: 50 - protein, 213 aa, synthetic construct
  REGION 1..213: note = Uliledlimab light chain
EIVLSQSPATLSLSPGERATLSCRASSRVNYMHWYQQKPGQSPRPWISATSNLASGVPARFSGSGSGTSYTLTISSLEPEDFAVYYCQQWSSNPPTFGGGTKVEIKRTVAAPSVFIFPPSDEQLKSGTASVVCLLNNFYPREAKVQWKVDNALQSGNSQESVTEQDSKDSTYSLSSTLTLSKADYEKHKVYACEVTHQGLSSPVTKSFNRGEC

SEQ ID NO: 51 - protein, 450 aa, synthetic construct
  REGION 1..450: note = BMS-986179 heavy chain
QVQLVESGGGVVQPGRSLRLSCAASGFTFSNYGMHWVRQAPGKGLEWVAVILYDGSNKYYPDSVKGRFTISRDNSKNTLYLQMNSLRAEDTAVYYCARGGSSWYPDSFDIWGQGTMVTVSSASTKGPSVFPLAPSSKSTSGGTAALGCLVKDYFPEPVTVSWNSGALTSGVHTFPAVLQSSGLYSLSSVVTVPSSSLGTQTYICNVNHKPSNTKVDKRVEPKSCDKTHTCPPCPAPEAAGGPSVFLFPPKPKDTLMISRTPEVTCVVVDVSHEDPEVKFNWYVDGVEVHNAKTKPREEQYNSTYRVVSVLTVLHQDWLNGKEYKCKVSNKALPAPIEKTISKAKGQPREPQVYTLPPSREEMTKNQVSLTCLVKGFYPSDIAVEWESNGQPENNYKTTPPVLDSDGSFFLYSKLTVDKSRWQQGNVFSCSVMHEALHNHYTQKSLSLSPG

SEQ ID NO: 52 - protein, 214 aa, synthetic construct
  REGION 1..214: note = BMS-986179 light chain
DIQMTQSPSSLSASVGDRVTITCRASQGISSWLAWYQQKPEKAPKSLIYAASSLQSGVPSRFSGSGSGTDFTLTISSLQPEDFATYYCQQYNSYPLTFGGGTKVEIKRTVAAPSVFIFPPSDEQLKSGTASVVCLLNNFYPREAKVQWKVDNALQSGNSQESVTEQDSKDSTYSLSSTLTLSKADYEKHKVYACEVTHQGLSSPVTKSFNRGEC

SEQ ID NO: 53 - protein, 121 aa, synthetic construct
  REGION 1..121: note = 900725 VH
QVQLVQSGAEVKKPGASVKLSCKASGYTFTSYWIHWVRQAPGQGLEWIGMIHPNSGSTYYNEKFKGRATLTVDKSTSTAYMELSSLRSEDTAVYYCARYYGSDYEWYFDVWGQGTTVTVSS

SEQ ID NO: 54 - protein, 107 aa, synthetic construct
  REGION 1..107: note = 900725 VL
DIQMTQSPSSMSASVGDRVTITCKASQNVRTAVVWYQQKPGKAPKALIYLASNRHTGVPDRFSGSGSGTDFTLTISSLQPEDFATYFCLQHWNYPYTFGQGTKLEIK